European Patent Application EP 4 480 493 A1, published December 25, 2024. Title: A RECOMBINANT HUMAN ALPHA-1 ANTITRYPSIN GLYCOPROTEIN FOR TREATING NON-VIRAL INFLAMMATORY DISEASES OF THE LUNG. Applicant: AATec Medical GmbH. The sequence listing filed with the application follows.

SEQUENCE LISTING (13 sequences)

SEQ ID NO: 1 - DNA, 1257 bp, Homo sapiens
  source 1..1257: mol_type = other DNA
atgccgtcttctgtctcgtggggcatcctcctgctggcaggcctgtgctgcctggtccctgtctccctggctgaggatccccagggagatgctgcccagaagacagatacatcccaccatgatcaggatcacccaaccttcaacaagatcacccccaacctggctgagttcgccttcagcctataccgccagctggcacaccagtccaacagcaccaatatcttcttctccccagtgagcatcgctacagcctttgcaatgctctccctggggaccaaggctgacactcacgatgaaatcctggagggcctgaatttcaacctcacggagattccggaggctcagatccatgaaggcttccaggaactcctccgtaccctcaaccagccagacagccagctccagctgaccaccggcaatggcctgttcctcagcgagggcctgaagctagtggataagtttttggaggatgttaaaaagttgtaccactcagaagccttcactgtcaacttcggggacaccgaagaggccaagaaacagatcaacgattacgtggagaagggtactcaagggaaaattgtggatttggtcaaggagcttgacagagacacagtttttgctctggtgaattacatcttctttaaaggcaaatgggagagaccctttgaagtcaaggacaccgaggaagaggacttccacgtggaccaggtgaccaccgtgaaggtgcctatgatgaagcgtttaggcatgtttaacatccagcactgtaagaagctgtccagctgggtgctgctgatgaaatacctgggcaatgccaccgccatcttcttcctgcctgatgaggggaaactacagcacctggaaaatgaactcacccacgatatcatcaccaagttcctggaaaatgaagacagaaggtctgccagcttacatttacccaaactgtccattactggaacctatgatctgaagagcgtcctgggtcaactgggcatcactaaggtcttcagcaatggggctgacctctccggggtcacagaggaggcacccctgaagctctccaaggccgtgcataaggctgtgctgaccatcgacgagaaagggactgaagctgctggggccatgtttttagaggccatacccatgtctatcccccccgaggtcaagttcaacaaaccctttgtcttcttaatgattgaacaaaataccaagtctcccctcttcatgggaaaagtggtgaatcccacccaaaaataa

SEQ ID NO: 2 - DNA, 1182 bp, Homo sapiens
  source 1..1182: mol_type = other DNA
gaagatccacaaggtgatgctgctcagaaaacagacacctcacaccatgatcaagatcatccgacatttaacaagatcacacctaaccttgcagagttcgccttttccttgtatcgtcagcttgctcatcaaagcaactcgacgaacattttcttttccccagtaagtattgcaactgcatttgctatgctatcgttgggtaccaaagctgacactcatgacgaaatattggagggtctaaactttaacttgacagaaatccccgaagcccaaattcatgagggatttcaagagttgttgagaactctaaaccaacctgactctcaactgcagttaactaccggtaatggactgttcttaagcgaaggtttaaaattggtcgataagttccttgaggacgttaagaagttgtatcactctgaggcttttacggtcaatttcggagatactgaggaagccaagaaacaaatcaatgactacgtggaaaagggaactcaaggcaagatcgttgacttggtgaaagaactggatagagataccgtatttgctttagtgaactacatcttctttaaagggaaatgggaaagaccattcgaggtcaaggatactgaggaggaagattttcacgtcgaccaggtaaccactgttaaggttccgatgatgaaacgattgggaatgttcaacattcagcactgtaagaagttgtcaagttgggttctgcttatgaagtacttagggaatgcaactgccattttcttcttgcctgatgaaggtaaactgcaacatttggaaaatgaacttacacacgatattatcaccaaatttctagagaacgaagataggagatcagcctctttgcatttgccaaagctgtcaataacaggtacttatgacttgaaatccgttcttggccaattgggcataactaaggtgttttctaatggtgctgatttgagtggtgttacagaggaagctcccttaaagctatctaaggctgttcacaaagcagttcttaccattgacgagaaaggtactgaagctgcaggagctatgtttctggaagccattcctatgtccattccacctgaagttaaattcaataagccttttgtctttcttatgattgagcagaatacgaaatctccattattcatgggaaaggtagtgaatccaacccagaaa

SEQ ID NO: 3 - DNA, 1188 bp, Homo sapiens
  source 1..1188: mol_type = other DNA
gaggaccctcaaggtgacgccgctcaaaagactgatacctcgcaccacgaccaagaccacccaacttttaacaagattactcctaatctagctgagttcgcattctctctctacagacaactcgctcatcagtctaactctacgaacattttcttctccccagtgtccattgcaactgctttcgccatgctttctttgggtactaaggctgacacacacgacgagattttagaaggattgaactttaatcttaccgaaattcctgaggcccaaattcacgaaggttttcaggagctgcttagaactcttaaccagccagatagccagctacaacttactactggaaatggactattcttgagtgaaggtctgaagctagttgacaaattcctcgaagatgtgaaaaagttgtaccattctgaggctttcaccgtcaacttcggtgacacagaggaggctaaaaagcagatcaacgactacgttgaaaagggtacgcaaggtaaaatcgttgacctcgttaaagagcttgatagagacaccgtatttgctcttgtcaattacatcttctttaaaggaaagtgggagagacctttcgaggtcaaggacaccgaggaggaagattttcatgtagatcaagtcaccactgttaaggttccaatgatgaagcgtctcggtatgtttaacatccaacactgtaaaaagctatcttcttgggtccttctgatgaagtacctgggtaacgctactgcaatcttcttcctaccagatgaaggtaagctccagcacctagagaacgaacttacccacgacatcattactaagttcctggaaaacgaagaccgtagatccgcttccctgcacctcccaaaactgtctatcactggtacctatgacctcaagtctgttctgggtcaactaggtataaccaaagtgttttcaaacggcgctgacctctccggtgtgactgaagaggcacctctcaagctgtccaaggccgttcacaaggcagtccttaccattgatgaaaagggaactgaagctgccggcgctatgttcctagaggccatcccaatgtcaattcctcccgaggttaagttcaacaagccattcgtcttcctaatgattgaacaaaacacaaagtctcctctgttcatgggaaaggttgttaacccaacccaaaagtaatag

SEQ ID NO: 4 - protein, 394 aa, Homo sapiens
EDPQGDAAQKTDTSHHDQDHPTFNKITPNLAEFAFSLYRQLAHQSNSTNIFFSPVSIATAFAMLSLGTKADTHDEILEGLNFNLTEIPEAQIHEGFQELLRTLNQPDSQLQLTTGNGLFLSEGLKLVDKFLEDVKKLYHSEAFTVNFGDTEEAKKQINDYVEKGTQGKIVDLVKELDRDTVFALVNYIFFKGKWERPFEVKDTEEEDFHVDQVTTVKVPMMKRLGMFNIQHCKKLSSWVLLMKYLGNATAIFFLPDEGKLQHLENELTHDIITKFLENEDRRSASLHLPKLSITGTYDLKSVLGQLGITKVFSNGADLSGVTEEAPLKLSKAVHKAVLTIDEKGTEAAGAMFLEAIPMSIPPEVKFNKPFVFLMIEQNTKSPLFMGKVVNPTQK

SEQ ID NO: 5 - DNA, 938 bp, Pichia pastoris
  source 1..938: mol_type = other DNA
agatctaacatccaaagacgaaaggttgaatgaaacctttttgccatccgacatccacaggtccattctcacacataagtgccaaacgcaacaggaggggatacactagcagcagaccgttgcaaacgcaggacctccactcctcttctcctcaacacccacttttgccatcgaaaaaccagcccagttattgggcttgattggagctcgctcattccaattccttctattaggctactaacaccatgactttattagcctgtctatcctggcccccctggcgaggttcatgtttgtttatttccgaatgcaacaagctccgcattacacccgaacatcactccagatgagggctttctgagtgtggggtcaaatagtttcatgttccccaaatggcccaaaactgacagtttaaacgctgtcttggaacctaatatgacaaaagcgtgatctcatccaagatgaactaagtttggttcgttgaaatgctaacggccagttggtcaaaaagaaacttccaaaagtcggcataccgtttgtcttgtttggtattgattgacgaatgctcaaaaataatctcattaatgcttagcgcagtctctctatcgcttctgaaccccggtgcacctgtgccgaaacgcaaatggggaaacacccgctttttggatgattatgcattgtctccacattgtatgcttccaagattctggtgggaatactgctgatagcctaacgttcatgatcaaaatttaactgttctaacccctacttgacagcaatatataaacagaaggaagctgccctgtcttaaacctttttttttatcatcattattagcttactttcataattgcgactggttccaattgacaagcttttgattttaacgacttttaacgacaacttgagaagatcaaaaaacaactaattattcgaaa

SEQ ID NO: 6 - protein, 30 aa, Homo sapiens
QLAHQSNSTNIFFSPVSIATAFAMLSLGTK

SEQ ID NO: 7 - protein, 30 aa, Homo sapiens; identical to SEQ ID NO: 6

SEQ ID NO: 8 - protein, 32 aa, Homo sapiens
ADTHDEILEGLNFNLTEIPEAQIHEGFQELLR

SEQ ID NO: 9 - protein, 11 aa, Homo sapiens
GLNFNLTEIPE

SEQ ID NO: 10 - protein, 16 aa, Homo sapiens
YLGNATAIFFLPDEGK

SEQ ID NO: 11 - protein, 16 aa, Homo sapiens
YLGNATAIFFLPDEGK

SEQ ID NO: 12 - protein, 21 aa, Homo sapiens
YLGNATAIFFLPDEGKLQHLE

SEQ ID NO: 13 - protein, 31 aa, Homo sapiens
YLGNATAIFFLPDEGKLQHLENELTHDIITK